European Patent Application EP 4 523 746 A1, published March 19, 2025. Title: Novel lactic acid bacteria and Compositions, food and beverages, and pharmaceuticals containing lactic acid bacteria. Applicant: MITSUBISHI GAS CHEMICAL COMPANY, INC. The sequence listing filed with the application follows.

SEQUENCE LISTING (10 sequences)

SEQ ID NO: 1 - DNA, 20 bp, synthetic construct
  misc_feature 1..20: note = Forward primer
  source 1..20: mol_type = other DNA
acaggaccatcggaatcttg

SEQ ID NO: 2 - DNA, 20 bp, synthetic construct
  misc_feature 1..20: note = Reverse primer
  source 1..20: mol_type = other DNA
cccttcttcaggtggaacac

SEQ ID NO: 3 - DNA, 21 bp, synthetic construct
  misc_feature 1..21: note = Forward primer
  source 1..21: mol_type = other DNA
tgtccaaggtggtaaagggtg

SEQ ID NO: 4 - DNA, 21 bp, synthetic construct
  misc_feature 1..21: note = Reverse primer
  source 1..21: mol_type = other DNA
ccggcgatttaactgatcctg

SEQ ID NO: 5 - DNA, 19 bp, synthetic construct
  misc_feature 1..19: note = Forward primer
  source 1..19: mol_type = other DNA
gaaggtgaaggtcggagtc

SEQ ID NO: 6 - DNA, 20 bp, synthetic construct
  misc_feature 1..20: note = Reverse primer
  source 1..20: mol_type = other DNA
gaagatggtgatgggatttc

SEQ ID NO: 7 - DNA, 21 bp, synthetic construct
  misc_feature 1..21: note = Forward primer
  source 1..21: mol_type = other DNA
accctgaaggtctgggagaaa

SEQ ID NO: 8 - DNA, 20 bp, synthetic construct
  misc_feature 1..20: note = Reverse primer
  source 1..20: mol_type = other DNA
ctgtggcctgaagctgtgta

SEQ ID NO: 9 - DNA, 22 bp, synthetic construct
  misc_feature 1..22: note = Forward primer
  source 1..22: mol_type = other DNA
atgagtatgctcaggctacaga

SEQ ID NO: 10 - DNA, 21 bp, synthetic construct
  misc_feature 1..21: note = Reverse primer
  source 1..21: mol_type = other DNA
gcattggcgatttcattggtc